European Patent Application EP 4 729 547 A1, published April 22, 2026. Title: ZINC FINGER PROTEIN, ZINC FINGER NUCLEASE, VECTOR, AND METHODS FOR GENOME EDITTING USING THEREOF. Applicant: VC GENE THERAPY. Application WO. The sequence listing filed with the application follows.

SEQUENCE LISTING (17 sequences)

SEQ ID NO: 1 - DNA, 18 bp, Mus musculus
  source 1..18: mol_type = genomic DNA
ctacgaagagcccgtggg

SEQ ID NO: 2 - DNA, 18 bp, Mus musculus
  source 1..18: mol_type = genomic DNA
accaaggctgcttggcga

SEQ ID NO: 3 - protein, 7 aa, synthetic construct
PKKKRKV

SEQ ID NO: 4 - protein, 27 aa, synthetic construct
PKKKRKVAAAPKKKRKVGSGPKKKRKV

SEQ ID NO: 5 - protein, 29 aa, synthetic construct
PKKKRKVAAAPAAKRVKLDGSGPKKKRKV

SEQ ID NO: 6 - protein, 7 aa, synthetic construct
PKKKRKV

SEQ ID NO: 7 - protein, 9 aa, synthetic construct
PAAKRVKLD

SEQ ID NO: 8 - protein, 17 aa, synthetic construct
KRXXXXXXXXXXKKKLD

SEQ ID NO: 9 - protein, 585 aa, Bacillus sp. SGD-V-76
MATKRVVRTFGWIQNPGKFENLKRTVQVFDENSKVYKEVRDIKIPNLVKDKDVRTTLIAAMNRLENYYSYKELVGTGTSVRAQAPCDAIIQAAIQDQGNKKGYIDNWSSDGFVRWAHALGFLEYNSDKDSFYLTDIGLEYSRSTDDSLNEKIILIEALSSYPPAIRILTLLENGEHLTKFDLGKQLGFSGESGFTSLPQNLFLDALANAPSSPPTIKNSIRSDWEGSADKYARMISGWLVKMGLVAQGRKNFVVPTVGGSTRNEYISHAFKITKDGLDVLRRAKGASKHVRVPKRVYWEMFATNINDRVYVRTRRAYTLYLLMRSNTALNTVQLQVKLKALGFEELEETIENDVKGLINSGIFINVTNKGYHFKDTIKPFEIPEFGVTEPLVKGEMEKKKSDLRHKLKHVPHEYIELIEIAQDSKQNRLFEFKVVEFLKEVYDYNGKHLGGSRKPDGALYTNGLKTDYGIILDTKAYKDGYSLPISQADEMQRYVDENNNRNAIINPNEWWKVYPNSILDFKFLFVSGFFKGDYKKQLARVSNLTKRKGAVLSVEQLLLGGEKIKDGSLTLEDVGDKFNNDEIIF

SEQ ID NO: 10 - DNA, 1758 bp, Bacillus sp. SGD-V-76
  source 1..1758: mol_type = other DNA
atggcaacaaaacgagtggttcgtacatttggttggatacagaatccaggtaaattcgagaacctaaaacgaacagtccaagtattcgatgaaaactcaaaagtatataaagaggttagggatataaagattccaaatctagtgaaagataaagatgtaagaactactttaatagctgctatgaatcgattagaaaattattactcatataaagagttggttggtacaggtacttcagttagagctcaagcgccttgtgatgccattattcaagcagcgattcaagaccaaggtaataaaaaaggatacattgataattggtcttctgatggattcgttcgttgggcacatgcattggggtttcttgagtataactcagataaggactcattttacctaactgatattggattggaatattctcgttctacagatgattcactaaatgaaaaaatcatacttattgaagcattgtcatcatatccaccagcaattcgaatattgacattacttgaaaatggtgagcatttaacaaaattcgacctaggtaaacagttaggctttagtggagagagtggttttacttcattaccacaaaacttatttttagatgcgttagcaaatgcaccttcatcaccaccaacaattaagaattctattcgttctgattgggaaggttctgcggataaatatgcacggatgatttcaggctggcttgtaaagatggggcttgttgcacaaggtcgtaaaaattttgttgtaccaacggtaggtggttctactcgaaatgagtatatatctcatgcttttaaaattacaaaagatggtcttgatgtgttaaggagagcaaaaggtgccagtaaacatgtacgagtaccaaagcgtgtatactgggagatgttcgctaccaacattaacgatagagtgtatgtaagaacaagacgggcttatacactttacttgttaatgagaagtaacactgctctaaatactgttcaacttcaagtgaaattaaaagctttgggctttgaagaattggaagaaacaattgagaatgatgtaaaaggtttaattaactctggaatttttatcaatgtgacgaataaaggttatcattttaaagatacaattaaaccattcgaaattcctgaatttggcgtaacagaaccattagtaaagggggaaatggagaagaagaaatccgatttgcgtcataagttaaaacacgtaccgcatgaatatattgaactaatagaaattgcacaggattcaaagcaaaatcgtttgttcgaatttaaagtagttgagtttttgaaagaagtttatgattataatggaaagcacctaggggggagtcgaaaaccagatggcgcactatataccaatggtttaaaaacagattatggaataattttagataccaaagcttacaaagatggttatagtttaccaatctcccaggcagatgaaatgcagcgttatgtcgatgaaaataataatagaaatgctattattaatcctaacgaatggtggaaagtgtatcctaattctatcttggactttaaattcttattcgtaagtggtttttttaaaggtgactataaaaaacaattagctcgtgtaagtaatcttacaaagcgtaaaggtgctgtcctaagcgtagagcaactattattgggaggggaaaaaattaaagatggtagtttaacattagaagatgttggtgacaaattcaataatgatgaaattattttctaa

SEQ ID NO: 11 - protein, 579 aa, Clostridium botulinum
VESLRLSDITIRTFGWIQNPSDFSKLKKIVQLFDHTSSIHVDLKENRIPRLVEKDDGRDRFIEILNRIPLKIKYIDLVGTSFKPRSSGRCNGIAQAMIEGQGKSFTDNWTADGFIRWAHALGFIQYDYLEDEFSITQAGFDFSRSINDSEGENEILIEAMLSYPPAVRVLDLLSLGEHLTKFDIGKNLGFNGESGFTSLPLNIMLQTLADNDLVSEKTKIRQDWEGSSDKYSRMIAGWLSKLGLVKKGKKYFDVNIGGIIHREYISHAYKITGEGLKQLRRAKGTTSARRIEKRVCWEMFATKNLDRTYIRTRRAYILKFLEVSSSLITIEQIKTKLLEKGYDETVETIKSDIKGLINIGLNIQETTRGYSLKDSINDFMIPVTDLNQIVKSSIEMSKANMRDNLQMLPHDYIELIEISQDPYQNRIFEMKVMDLFINEYGFSGSHLGGSRKPDGAMYAHGFGVIVDTKAYKDGYNLPISQADEMERYVRENIDRNEHVNSNRWWNIFPEDTNEYKFLFVSGFFKGNFEKQLERISIDTGVQGGALSVEHLLLGAEYIKRGILTLYDFKNSFLNKEIQF

SEQ ID NO: 12 - DNA, 1740 bp, Clostridium botulinum
  source 1..1740: mol_type = other DNA
gtggaatcattaagattatcagacataacaattagaacatttgggtggattcagaatcctagtgattttagtaaattaaaaaaaatagttcagttatttgatcatacatcatctattcatgtggatttgaaagaaaaccgcataccacggttagtggagaaagatgacggacgtgataggtttattgagatattaaatcggattccgttaaagataaagtatattgatttagtaggaacatcatttaaacctagaagtagtggtagatgtaatggaattgctcaagcaatgattgaaggtcaaggtaagagttttactgataattggacagctgatgggtttattaggtgggctcatgcacttggctttatacaatatgattatttagaagatgagttttcaataacacaagcaggctttgatttttcaaggtcaatcaatgatagtgaaggggaaaatgaaatattaatagaggcaatgttgtcttatccacctgcagttagagttttagatttactttctttaggagagcatcttacaaaatttgatattggaaaaaatctgggcttcaatggcgaatcaggatttacatctttacctttaaatatcatgcttcaaacattagcagacaatgatttagtaagtgaaaagactaaaattcgtcaggattgggaaggttcttctgataagtattcacgaatgatagccggctggttatcgaaacttggtttggttaaaaagggaaaaaagtattttgatgtaaatattggaggaataattcatagagaatatatctctcatgcatataaaattactggagaaggtttaaaacaactccgtagggctaaaggaactacaagtgcaaggcgtatagaaaaacgggtttgctgggaaatgttcgccacaaagaatctagataggacatatattcgtacaagaagagcttatattttaaagtttttagaagtttcaagcagcttaattactattgagcaaattaagactaagttattggaaaaaggttatgacgaaacagtagaaactattaaatctgatattaaggggttaattaacattggtttaaatattcaagaaaccactcgaggttattcattaaaggattcaattaatgactttatgattccagtaaccgacttaaatcaaattgttaaaagtagtatagagatgtctaaagctaacatgagagacaatcttcagatgttgcctcatgattatattgagctaattgaaatatcacaagatccatatcaaaatagaatatttgaaatgaaagttatggatttatttattaatgagtatggtttcagtggttcgcacttaggtggaagtaggaaacctgatggtgctatgtatgcacatggttttggtgttattgttgatacaaaagcatataaagatgggtacaatcttcctataagtcaagctgatgaaatggaacgatatgtaagggaaaatattgatagaaatgaacatgtgaactcaaatagatggtggaatatatttcccgaagatacaaatgaatataagtttttattcgtaagtggtttctttaaaggaaattttgagaaacaattagaaaggataagtatagatactggtgtacaaggaggggctttaagtgttgaacatttattattaggtgctgagtacataaagaggggtattcttactttatatgattttaagaatagctttttaaataaggaaattcaattttaa

SEQ ID NO: 13 - protein, 4 aa, synthetic construct
TGGS

SEQ ID NO: 14 - protein, 195 aa, synthetic construct
LVKGEMEKKKSDLRHKLKHVPHEYIELIEIAQDSKQNRLFEFKVVEFLKEVYDYNGKHLGGSRKPDGALYTNGLKTDYGIILDTKAYKDGYSLPISQADEMQDYVDENNNRDAIINPNEWWKVYPNSILDFKFLFVSGFFKGDYKKQLARVSNLTKRKGAVLSVEQLLLGGEKIKDGSLTLEDVGDKFNNDEIIF

SEQ ID NO: 15 - protein, 195 aa, synthetic construct
LVKGEMEKKKSDLRHKLKHVPHEYIELIEIAQDSKQNRLFEFKVVEFLKEVYDYNGKHLGGSRKPDGALYTNGLKTDYGIILDTKAYKDGYSLPISQAREMQRYVDENNNRNAIINPNEWWKVYPNSILDFKFLFVSGFFKGDYKKQLARVSRLTKRKGAVLSVEQLLLGGEKIKDGSLTLEDVGDKFNNDEIIF

SEQ ID NO: 16 - protein, 367 aa, synthetic construct
PGEKPYKCPECGKSFSRSDKLVRHQRTHTGEKPYKCPECGKSFSSRRTCRAHQRTHTGEKPYKCPECGKSFSDCRDLARHQRTHTGEKPYKCPECGKSFSQLAHLRAHQRTHTGEKPYKCPECGKSFSQSGHLTEHQRTHTGEKPYKCPECGKSFSQNSTLTEHQRTHTGGSLVKGEMEKKKSDLRHKLKHVPHEYIELIEIAQDSKQNRLFEFKVVEFLKEVYDYNGKHLGGSRKPDGALYTNGLKTDYGIILDTKAYKDGYSLPISQADEMQDYVDENNNRDAIINPNEWWKVYPNSILDFKFLFVSGFFKGDYKKQLARVSNLTKRKGAVLSVEQLLLGGEKIKDGSLTLEDVGDKFNNDEIIF

SEQ ID NO: 17 - protein, 367 aa, synthetic construct
PGEKPYKCPECGKSFSQSGHLTEHQRTHTGEKPYKCPECGKSFSRSDHLTTHQRTHTGEKPYKCPECGKSFSTSGELVRHQRTHTGEKPYKCPECGKSFSTSGELVRHQRTHTGEKPYKCPECGKSFSRKDNLKNHQRTHTGEKPYKCPECGKSFSDKKDLTRHQRTHTGGSLVKGEMEKKKSDLRHKLKHVPHEYIELIEIAQDSKQNRLFEFKVVEFLKEVYDYNGKHLGGSRKPDGALYTNGLKTDYGIILDTKAYKDGYSLPISQAREMQRYVDENNNRNAIINPNEWWKVYPNSILDFKFLFVSGFFKGDYKKQLARVSRLTKRKGAVLSVEQLLLGGEKIKDGSLTLEDVGDKFNNDEIIF